European Patent Specification EP 3 495 383 B1, published March 29, 2023. Title: PEPTIDE SHOWIG MELANIN GENERATION-PROMOTING ACTIVITY, AND USE THEREOF. Applicant: CAREGEN CO., LTD. The sequence listing filed with the application follows.

SEQUENCE LISTING (8 sequences)

SEQ ID NO: 1 - protein, 8 aa, Artificial Sequence
  Synthetic Construct
RWRRKIEN

SEQ ID NO: 2 - protein, 12 aa, Artificial Sequence
  Synthetic Construct
FCLGPCPYIWSL

SEQ ID NO: 3 - DNA, 21 bp, MITF Forward Primer
ccagcctggcgatcatgtcat

SEQ ID NO: 4 - DNA, 20 bp, MITF Reverse Primer
ggtctggacaggagttgctg

SEQ ID NO: 5 - DNA, 20 bp, Tyrosinase Forward Primer
ggccagctttcaggcagagg

SEQ ID NO: 6 - DNA, 20 bp, Tyrosinase Reverse Primer
tggtgcttcatgggcaaaat

SEQ ID NO: 7 - DNA, 20 bp, TRP1 Forward Primer
tctgtgaaggtgtgcaggag

SEQ ID NO: 8 - DNA, 20 bp, TRP1 Reverse Primer
ccgaaacagagtggaaggtt